European Patent Application EP 4 640 833 A1, published October 29, 2025. Title: 一种猴痘病毒核酸疫苗及其用途. Applicant: 中国科学院微生物研究所. The sequence listing filed with the application follows.

SEQUENCE LISTING (19 sequences)

SEQ ID NO: 1 - protein, 92 aa, synthetic construct
STTQYDHKESCNGLYYQGSCYILHSDYKSFEDAKANCAAESSTLPNKSDVLTTWLIDYVEDTWGSDGNPITKTTSDYQDSDVSQEVRKYFCT

SEQ ID NO: 2 - protein, 118 aa, synthetic construct
SANKAAITDSAVAVAAASSTHRKVVSSTTQYDHKESCNGLYYQGSCYILHSDYKSFEDAKANCAAESSTLPNKSDVLTTWLIDYVEDTWGSDGNPITKTTSDYQDSDVSQEVRKYFCT

SEQ ID NO: 3 - protein, 179 aa, synthetic construct
AAASIQTTVNTLSERISSKLEQEANASAQTKCDIEIGNFYIRQNHGCNITVKNMCSADADAQLDAVLSAATETYSGLTPEQKAYVPAMFTAALNIQTSVNTVVRDFENYVKQTCNSSAVVDNKLKIQNVIIDECYGAPGSPTNLEFINTGSSKGNCAIKALMQLTTKATTQIAPRQVAG

SEQ ID NO: 4 - DNA, 276 bp, synthetic construct
  source 1..276: mol_type = other DNA
agcaccacccagtacgaccacaaagagagctgcaacggcctgtactaccaaggctcttgttacatcctgcacagcgactataagagcttcgaggatgctaaggccaattgcgccgccgagagcagcacactgcctaacaagtccgacgtgctgaccacctggctgatcgactacgtggaagatacatggggaagcgacggcaaccccatcacaaaaaccacaagcgattatcaggacagcgacgtgtctcaggaggttagaaagtacttttgcacc

SEQ ID NO: 5 - DNA, 354 bp, synthetic construct
  source 1..354: mol_type = other DNA
tccgccaataaggcagccatcaccgactctgccgtggcagtggcagcagccagctccacacaccgcaaggtggtgtctagcaccacacagtacgatcacaaggaatcctgtaatggcctgtactatcagggctcctgttacatcctgcactctgactataagagctttgaggatgccaaggccaactgtgccgccgagtcctctaccctgccaaataagagcgacgtgctgaccacatggctgatcgactatgtggaggatacctggggctctgatggcaaccccatcacaaagaccacatctgattaccaggacagcgacgtgagccaggaggtgcggaagtatttctgcacc

SEQ ID NO: 6 - RNA, 276 nt, synthetic construct
  source 1..276: mol_type = other RNA
agcaccacccagtacgaccacaaagagagctgcaacggcctgtactaccaaggctcttgttacatcctgcacagcgactataagagcttcgaggatgctaaggccaattgcgccgccgagagcagcacactgcctaacaagtccgacgtgctgaccacctggctgatcgactacgtggaagatacatggggaagcgacggcaaccccatcacaaaaaccacaagcgattatcaggacagcgacgtgtctcaggaggttagaaagtacttttgcacc

SEQ ID NO: 7 - RNA, 354 nt, synthetic construct
  source 1..354: mol_type = other RNA
tccgccaataaggcagccatcaccgactctgccgtggcagtggcagcagccagctccacacaccgcaaggtggtgtctagcaccacacagtacgatcacaaggaatcctgtaatggcctgtactatcagggctcctgttacatcctgcactctgactataagagctttgaggatgccaaggccaactgtgccgccgagtcctctaccctgccaaataagagcgacgtgctgaccacatggctgatcgactatgtggaggatacctggggctctgatggcaaccccatcacaaagaccacatctgattaccaggacagcgacgtgagccaggaggtgcggaagtatttctgcacc

SEQ ID NO: 8 - DNA, 537 bp, synthetic construct
  source 1..537: mol_type = other DNA
gccgccgcctctatccagaccacagtgaacaccctgagcgagcggatcagctccaagctggagcaggaggcaaacgcaagcgcccagacaaagtgcgacatcgagatcggcaatttctacatcagacagaaccacggctgcaatatcaccgtgaagaatatgtgctccgccgacgcagatgcacagctggatgccgtgctgtccgccgcaaccgagacatactctggcctgacccctgagcagaaggcctatgtgccagccatgttcacagccgccctgaacatccagaccagcgtgaatacagtggtgcgggactttgagaactacgtgaagcagacctgcaattctagcgccgtggtggacaacaagctgaagatccagaatgtgatcatcgatgagtgttatggagcaccaggctcccctaccaacctggagttcatcaatacaggctcctctaagggcaactgcgccatcaaggccctgatgcagctgaccacaaaggccaccacacagatcgcacctaggcaggtggcaggc

SEQ ID NO: 9 - RNA, 537 nt, synthetic construct
  source 1..537: mol_type = other RNA
gccgccgcctctatccagaccacagtgaacaccctgagcgagcggatcagctccaagctggagcaggaggcaaacgcaagcgcccagacaaagtgcgacatcgagatcggcaatttctacatcagacagaaccacggctgcaatatcaccgtgaagaatatgtgctccgccgacgcagatgcacagctggatgccgtgctgtccgccgcaaccgagacatactctggcctgacccctgagcagaaggcctatgtgccagccatgttcacagccgccctgaacatccagaccagcgtgaatacagtggtgcgggactttgagaactacgtgaagcagacctgcaattctagcgccgtggtggacaacaagctgaagatccagaatgtgatcatcgatgagtgttatggagcaccaggctcccctaccaacctggagttcatcaatacaggctcctctaagggcaactgcgccatcaaggccctgatgcagctgaccacaaaggccaccacacagatcgcacctaggcaggtggcaggc

SEQ ID NO: 10 - protein, 542 aa, synthetic construct
STTQYDHKESCNGLYYQGSCYILHSDYKSFEDAKANCAAESSTLPNKSDVLTTWLIDYVEDTWGSDGNPITKTTSDYQDSDVSQEVRKYFCTAAASIQTTVNTLSERISSKLEQEANASAQTKCDIEIGNFYIRQNHGCNITVKNMCSADADAQLDAVLSAATETYSGLTPEQKAYVPAMFTAALNIQTSVNTVVRDFENYVKQTCNSSAVVDNKLKIQNVIIDECYGAPGSPTNLEFINTGSSKGNCAIKALMQLTTKATTQIAPRQVAGSTTQYDHKESCNGLYYQGSCYILHSDYKSFEDAKANCAAESSTLPNKSDVLTTWLIDYVEDTWGSDGNPITKTTSDYQDSDVSQEVRKYFCTAAASIQTTVNTLSERISSKLEQEANASAQTKCDIEIGNFYIRQNHGCNITVKNMCSADADAQLDAVLSAATETYSGLTPEQKAYVPAMFTAALNIQTSVNTVVRDFENYVKQTCNSSAVVDNKLKIQNVIIDECYGAPGSPTNLEFINTGSSKGNCAIKALMQLTTKATTQIAPRQVAG

SEQ ID NO: 11 - protein, 568 aa, synthetic construct
STTQYDHKESCNGLYYQGSCYILHSDYKSFEDAKANCAAESSTLPNKSDVLTTWLIDYVEDTWGSDGNPITKTTSDYQDSDVSQEVRKYFCTAAASIQTTVNTLSERISSKLEQEANASAQTKCDIEIGNFYIRQNHGCNITVKNMCSADADAQLDAVLSAATETYSGLTPEQKAYVPAMFTAALNIQTSVNTVVRDFENYVKQTCNSSAVVDNKLKIQNVIIDECYGAPGSPTNLEFINTGSSKGNCAIKALMQLTTKATTQIAPRQVAGSANKAAITDSAVAVAAASSTHRKVVSSTTQYDHKESCNGLYYQGSCYILHSDYKSFEDAKANCAAESSTLPNKSDVLTTWLIDYVEDTWGSDGNPITKTTSDYQDSDVSQEVRKYFCTAAASIQTTVNTLSERISSKLEQEANASAQTKCDIEIGNFYIRQNHGCNITVKNMCSADADAQLDAVLSAATETYSGLTPEQKAYVPAMFTAALNIQTSVNTVVRDFENYVKQTCNSSAVVDNKLKIQNVIIDECYGAPGSPTNLEFINTGSSKGNCAIKALMQLTTKATTQIAPRQVAG

SEQ ID NO: 12 - DNA, 1626 bp, synthetic construct
  source 1..1626: mol_type = other DNA
agcaccacccagtacgaccacaaagagagctgcaacggcctgtactaccaaggctcttgttacatcctgcacagcgactataagagcttcgaggatgctaaggccaattgcgccgccgagagcagcacactgcctaacaagtccgacgtgctgaccacctggctgatcgactacgtggaagatacatggggaagcgacggcaaccccatcacaaaaaccacaagcgattatcaggacagcgacgtgtctcaggaggttagaaagtacttttgcaccgccgccgcctctatccagaccacagtgaacaccctgagcgagcggatcagctccaagctggagcaggaggcaaacgcaagcgcccagacaaagtgcgacatcgagatcggcaatttctacatcagacagaaccacggctgcaatatcaccgtgaagaatatgtgctccgccgacgcagatgcacagctggatgccgtgctgtccgccgcaaccgagacatactctggcctgacccctgagcagaaggcctatgtgccagccatgttcacagccgccctgaacatccagaccagcgtgaatacagtggtgcgggactttgagaactacgtgaagcagacctgcaattctagcgccgtggtggacaacaagctgaagatccagaatgtgatcatcgatgagtgttatggagcaccaggctcccctaccaacctggagttcatcaatacaggctcctctaagggcaactgcgccatcaaggccctgatgcagctgaccacaaaggccaccacacagatcgcacctaggcaggtggcaggcagcaccacacagtacgatcacaaggaatcctgtaatggcctgtactatcagggctcctgttacatcctgcactctgactataagagctttgaggatgccaaggccaactgtgccgccgagtcctctaccctgccaaataagagcgacgtgctgaccacatggctgatcgactatgtggaggatacctggggctctgatggcaaccccatcacaaagaccacatctgattaccaggacagcgacgtgagccaggaggtgcggaagtatttctgcaccgctgctgcttccatccagaccacagtgaatacactgagcgagagaatcagctccaaactggagcaggaggccaacgcctctgcccagaccaagtgtgacatcgagatcggcaacttctacatcaggcagaatcatggatgtaatatcaccgtgaagaacatgtgctccgccgatgccgacgcccagctggacgccgtgctgagcgccgccactgagacatactccggcctgacccccgaacagaaagcctatgtgcctgctatgtttaccgccgccctgaacattcagaccagcgtcaacacagtggtgcgcgatttcgaaaattatgtcaaacagacttgtaattctagcgccgtcgtcgataacaagctgaagattcagaatgtgattattgacgaatgctacggagcaccaggctccccaaccaacctggagtttatcaacaccggctcctctaagggcaattgtgccatcaaggccctgatgcaactgactaccaaagctaccacacagatcgcaccaaggcaggtggcagga

SEQ ID NO: 13 - DNA, 1704 bp, synthetic construct
  source 1..1704: mol_type = other DNA
agcaccacccagtacgaccacaaagagagctgcaacggcctgtactaccaaggctcttgttacatcctgcacagcgactataagagcttcgaggatgctaaggccaattgcgccgccgagagcagcacactgcctaacaagtccgacgtgctgaccacctggctgatcgactacgtggaagatacatggggaagcgacggcaaccccatcacaaaaaccacaagcgattatcaggacagcgacgtgtctcaggaggttagaaagtacttttgcaccgccgccgcctctatccagaccacagtgaacaccctgagcgagcggatcagctccaagctggagcaggaggcaaacgcaagcgcccagacaaagtgcgacatcgagatcggcaatttctacatcagacagaaccacggctgcaatatcaccgtgaagaatatgtgctccgccgacgcagatgcacagctggatgccgtgctgtccgccgcaaccgagacatactctggcctgacccctgagcagaaggcctatgtgccagccatgttcacagccgccctgaacatccagaccagcgtgaatacagtggtgcgggactttgagaactacgtgaagcagacctgcaattctagcgccgtggtggacaacaagctgaagatccagaatgtgatcatcgatgagtgttatggagcaccaggctcccctaccaacctggagttcatcaatacaggctcctctaagggcaactgcgccatcaaggccctgatgcagctgaccacaaaggccaccacacagatcgcacctaggcaggtggcaggctccgccaataaggcagccatcaccgactctgccgtggcagtggcagcagccagctccacacaccgcaaggtggtgtctagcaccacacagtacgatcacaaggaatcctgtaatggcctgtactatcagggctcctgttacatcctgcactctgactataagagctttgaggatgccaaggccaactgtgccgccgagtcctctaccctgccaaataagagcgacgtgctgaccacatggctgatcgactatgtggaggatacctggggctctgatggcaaccccatcacaaagaccacatctgattaccaggacagcgacgtgagccaggaggtgcggaagtatttctgcaccgctgctgcttccatccagaccacagtgaatacactgagcgagagaatcagctccaaactggagcaggaggccaacgcctctgcccagaccaagtgtgacatcgagatcggcaacttctacatcaggcagaatcatggatgtaatatcaccgtgaagaacatgtgctccgccgatgccgacgcccagctggacgccgtgctgagcgccgccactgagacatactccggcctgacccccgaacagaaagcctatgtgcctgctatgtttaccgccgccctgaacattcagaccagcgtcaacacagtggtgcgcgatttcgaaaattatgtcaaacagacttgtaattctagcgccgtcgtcgataacaagctgaagattcagaatgtgattattgacgaatgctacggagcaccaggctccccaaccaacctggagtttatcaacaccggctcctctaagggcaattgtgccatcaaggccctgatgcaactgactaccaaagctaccacacagatcgcaccaaggcaggtggcagga

SEQ ID NO: 14 - RNA, 1626 nt, synthetic construct
  source 1..1626: mol_type = other RNA
agcaccacccagtacgaccacaaagagagctgcaacggcctgtactaccaaggctcttgttacatcctgcacagcgactataagagcttcgaggatgctaaggccaattgcgccgccgagagcagcacactgcctaacaagtccgacgtgctgaccacctggctgatcgactacgtggaagatacatggggaagcgacggcaaccccatcacaaaaaccacaagcgattatcaggacagcgacgtgtctcaggaggttagaaagtacttttgcaccgccgccgcctctatccagaccacagtgaacaccctgagcgagcggatcagctccaagctggagcaggaggcaaacgcaagcgcccagacaaagtgcgacatcgagatcggcaatttctacatcagacagaaccacggctgcaatatcaccgtgaagaatatgtgctccgccgacgcagatgcacagctggatgccgtgctgtccgccgcaaccgagacatactctggcctgacccctgagcagaaggcctatgtgccagccatgttcacagccgccctgaacatccagaccagcgtgaatacagtggtgcgggactttgagaactacgtgaagcagacctgcaattctagcgccgtggtggacaacaagctgaagatccagaatgtgatcatcgatgagtgttatggagcaccaggctcccctaccaacctggagttcatcaatacaggctcctctaagggcaactgcgccatcaaggccctgatgcagctgaccacaaaggccaccacacagatcgcacctaggcaggtggcaggcagcaccacacagtacgatcacaaggaatcctgtaatggcctgtactatcagggctcctgttacatcctgcactctgactataagagctttgaggatgccaaggccaactgtgccgccgagtcctctaccctgccaaataagagcgacgtgctgaccacatggctgatcgactatgtggaggatacctggggctctgatggcaaccccatcacaaagaccacatctgattaccaggacagcgacgtgagccaggaggtgcggaagtatttctgcaccgctgctgcttccatccagaccacagtgaatacactgagcgagagaatcagctccaaactggagcaggaggccaacgcctctgcccagaccaagtgtgacatcgagatcggcaacttctacatcaggcagaatcatggatgtaatatcaccgtgaagaacatgtgctccgccgatgccgacgcccagctggacgccgtgctgagcgccgccactgagacatactccggcctgacccccgaacagaaagcctatgtgcctgctatgtttaccgccgccctgaacattcagaccagcgtcaacacagtggtgcgcgatttcgaaaattatgtcaaacagacttgtaattctagcgccgtcgtcgataacaagctgaagattcagaatgtgattattgacgaatgctacggagcaccaggctccccaaccaacctggagtttatcaacaccggctcctctaagggcaattgtgccatcaaggccctgatgcaactgactaccaaagctaccacacagatcgcaccaaggcaggtggcagga

SEQ ID NO: 15 - RNA, 1704 nt, synthetic construct
  source 1..1704: mol_type = other RNA
agcaccacccagtacgaccacaaagagagctgcaacggcctgtactaccaaggctcttgttacatcctgcacagcgactataagagcttcgaggatgctaaggccaattgcgccgccgagagcagcacactgcctaacaagtccgacgtgctgaccacctggctgatcgactacgtggaagatacatggggaagcgacggcaaccccatcacaaaaaccacaagcgattatcaggacagcgacgtgtctcaggaggttagaaagtacttttgcaccgccgccgcctctatccagaccacagtgaacaccctgagcgagcggatcagctccaagctggagcaggaggcaaacgcaagcgcccagacaaagtgcgacatcgagatcggcaatttctacatcagacagaaccacggctgcaatatcaccgtgaagaatatgtgctccgccgacgcagatgcacagctggatgccgtgctgtccgccgcaaccgagacatactctggcctgacccctgagcagaaggcctatgtgccagccatgttcacagccgccctgaacatccagaccagcgtgaatacagtggtgcgggactttgagaactacgtgaagcagacctgcaattctagcgccgtggtggacaacaagctgaagatccagaatgtgatcatcgatgagtgttatggagcaccaggctcccctaccaacctggagttcatcaatacaggctcctctaagggcaactgcgccatcaaggccctgatgcagctgaccacaaaggccaccacacagatcgcacctaggcaggtggcaggctccgccaataaggcagccatcaccgactctgccgtggcagtggcagcagccagctccacacaccgcaaggtggtgtctagcaccacacagtacgatcacaaggaatcctgtaatggcctgtactatcagggctcctgttacatcctgcactctgactataagagctttgaggatgccaaggccaactgtgccgccgagtcctctaccctgccaaataagagcgacgtgctgaccacatggctgatcgactatgtggaggatacctggggctctgatggcaaccccatcacaaagaccacatctgattaccaggacagcgacgtgagccaggaggtgcggaagtatttctgcaccgctgctgcttccatccagaccacagtgaatacactgagcgagagaatcagctccaaactggagcaggaggccaacgcctctgcccagaccaagtgtgacatcgagatcggcaacttctacatcaggcagaatcatggatgtaatatcaccgtgaagaacatgtgctccgccgatgccgacgcccagctggacgccgtgctgagcgccgccactgagacatactccggcctgacccccgaacagaaagcctatgtgcctgctatgtttaccgccgccctgaacattcagaccagcgtcaacacagtggtgcgcgatttcgaaaattatgtcaaacagacttgtaattctagcgccgtcgtcgataacaagctgaagattcagaatgtgattattgacgaatgctacggagcaccaggctccccaaccaacctggagtttatcaacaccggctcctctaagggcaattgtgccatcaaggccctgatgcaactgactaccaaagctaccacacagatcgcaccaaggcaggtggcagga

SEQ ID NO: 16 - DNA, 47 bp, synthetic construct
  source 1..47: mol_type = other DNA
gggaaataagagagaaaagaagagtaagaagaaatataagagccacc

SEQ ID NO: 17 - protein, 20 aa, synthetic construct
METDTLLLWVLLLWVPGSTG

SEQ ID NO: 18 - DNA, 60 bp, synthetic construct
  source 1..60: mol_type = other DNA
atggaaacagacaccctgctgctgtgggtcctgctgctctgggtgcctggcagcaccggc

SEQ ID NO: 19 - DNA, 110 bp, synthetic construct
  source 1..110: mol_type = other DNA
tgataataggctggagcctcggtggccatgcttcttgccccttgggcctccccccagcccctcctccccttcctgcacccgtacccccgtggtctttgaataaagtctga